European Patent Application EP 4 596 681 A1, published August 6, 2025. Title: Human astrocyte cell population, cell population culture, method for producing human astrocyte cell population, and method for evaluating test substance. Applicant: FUJIFILM Corporation. Application WO. The sequence listing filed with the application follows.

SEQUENCE LISTING (10 sequences)

SEQ ID NO: 1 - DNA, 20 bp, synthetic construct
  source 1..20: mol_type = other DNA
cacattcatgtgggcatttc

SEQ ID NO: 2 - DNA, 23 bp, synthetic construct
  source 1..23: mol_type = other DNA
agctttggttctgccatttgcta

SEQ ID NO: 3 - DNA, 20 bp, synthetic construct
  source 1..20: mol_type = other DNA
ttgcctcaacgaaaagagct

SEQ ID NO: 4 - DNA, 20 bp, synthetic construct
  source 1..20: mol_type = other DNA
cggtccttcttcactgcttc

SEQ ID NO: 5 - DNA, 20 bp, synthetic construct
  source 1..20: mol_type = other DNA
tggccccactatctatcagc

SEQ ID NO: 6 - DNA, 20 bp, synthetic construct
  source 1..20: mol_type = other DNA
tggacccttgactctgttcc

SEQ ID NO: 7 - DNA, 20 bp, synthetic construct
  source 1..20: mol_type = other DNA
gtgagacttgcctgctcctc

SEQ ID NO: 8 - DNA, 20 bp, synthetic construct
  source 1..20: mol_type = other DNA
cgtcccgttgaagaaatgac

SEQ ID NO: 9 - DNA, 22 bp, synthetic construct
  source 1..22: mol_type = other DNA
gtggaaatccgagccgttctct

SEQ ID NO: 10 - DNA, 22 bp, synthetic construct
  source 1..22: mol_type = other DNA
gatggttacggtctgctggtga